European Patent Specification EP 3 529 616 B1, published September 6, 2023. Title: IN VITRO AND CELL BASED ASSAYS FOR MEASURING THE ACTIVITY OF BOTULINUM NEUROTOXINS. Applicant: PRESIDENT AND FELLOWS OF HARVARD COLLEGE. The sequence listing filed with the application follows.

SEQUENCE LISTING (32 sequences)

SEQ ID NO: 1 - protein, 170 aa, Artificial Sequence
  source: /note="Description of Artificial Sequence: Synthetic polypeptide"
MVFTLEDFVGDWEQTAAYNLDQVLEQGGVSSLLQNLAVSVTPIQRIVRSGENALKIDIHVIIPYEGLSADQMAQIEEVFKVVYPVDDHHFKVILPYGTLVIDGVTPNMLNYFGRPYEGIAVFDGKKITVTGTLWNGNKIIDERLITPDGSMLFRVTINSVTGYRLFEEIL

SEQ ID NO: 2 - protein, 159 aa, Artificial Sequence
  source: /note="Description of Artificial Sequence: Synthetic polypeptide"
MVFTLEDFVGDWEQTAAYNLDQVLEQGGVSSLLQNLAVSVTPIQRIVRSGENALKIDIHVIIPYEGLSADQMAQIEEVFKVVYPVDDHHFKVILPYGTLVIDGVTPNMLNYFGRPYEGIAVFDGKKITVTGTLWNGNKIIDERLITPDGSMLFRVTINS

SEQ ID NO: 3 - protein, 11 aa, Artificial Sequence
  source: /note="Description of Artificial Sequence: Synthetic peptide"
VTGYRLFEEIL

SEQ ID NO: 4 - protein, 15 aa, Artificial Sequence
  source: /note="Description of Artificial Sequence: Synthetic peptide"
GSSGGGGSGGGGSSG

SEQ ID NO: 5 - protein, 14 aa, Artificial Sequence
  source: /note="Description of Artificial Sequence: Synthetic peptide"
GSSGGGGSGGGSSG

SEQ ID NO: 6 - protein, 5 aa, Artificial Sequence
  source: /note="Description of Artificial Sequence: Synthetic peptide"
GGGGS

SEQ ID NO: 7 - protein, 15 aa, Artificial Sequence
  source: /note="Description of Artificial Sequence: Synthetic peptide"
  MISC_FEATURE (1)..(15): /note="This sequence may encompass 1-3 'Gly Gly Gly Gly Ser' repeating units"
GGGGSGGGGSGGGGS

SEQ ID NO: 8 - protein, 18 aa, Artificial Sequence
  source: /note="Description of Artificial Sequence: Synthetic peptide"
KESGSVSSEQLAQFRSLD

SEQ ID NO: 9 - protein, 14 aa, Artificial Sequence
  source: /note="Description of Artificial Sequence: Synthetic peptide"
EGKSSGSGSESKST

SEQ ID NO: 10 - protein, 66 aa, Unknown
  source: /note="Description of Unknown: Human or rat SNAP25b polypeptide"
ARENEMDENLEQVSGIIGNLRHMALDMGNEIDTQNRQIDRIMEKADSNKTRIDEANQRATKMLGSG

SEQ ID NO: 11 - protein, 38 aa, Homo sapiens
NTYFKNCTFIDTVFDNTDFEPYKFIDSEFKNCSFFHNK

SEQ ID NO: 12 - protein, 6 aa, Artificial Sequence
  source: /note="Description of Artificial Sequence: Synthetic 6xHis tag"
HHHHHH

SEQ ID NO: 13 - protein, 550 aa, Photinus pyralis
MEDAKNIKKGPAPFYPLEDGTAGEQLHKAMKRYALVPGTIAFTDAHIEVDITYAEYFEMSVRLAEAMKRYGLNTNHRIVVCSENSLQFFMPVLGALFIGVAVAPANDIYNERELLNSMGISQPTVVFVSKKGLQKILNVQKKLPIIQKIIIMDSKTDYQGFQSMYTFVTSHLPPGFNEYDFVPESFDRDKTIALIMNSSGSTGLPKGVALPHRTACVRFSHARDPIFGNQIIPDTAILSVVPFHHGFGMFTTLGYLICGFRVVLMYRFEEELFLRSLQDYKIQSALLVPTLFSFFAKSTLIDKYDLSNLHEIASGGAPLSKEVGEAVAKRFHLPGIRQGYGLTETTSAILITPEGDDKPGAVGKVVPFFEAKVVDLDTGKTLGVNQRGELCVRGPMIMSGYVNNPEATNALIDKDGWLHSGDIAYWDEDEHFFIVDRLKSLIKYKGYQVAPAELESILLQHPNIFDAGVAGLPDDDAGELPAAVVVLEHGKTMTEKEIVDYVASQVTTAKKLRGGVVFVDEVPKGLTGKLDARKIREILIKAKKGGKIAV

SEQ ID NO: 14 - protein, 206 aa, Homo sapiens
MAEDADMRNELEEMQRRADQLADESLESTRRMLQLVEESKDAGIRTLVMLDEQGEQLERIEEGMDQINKDMKEAEKNLTDLGKFCGLCVCPCNKLKSSDAYKKAWGNNQDGVVASQPARVVDEREQMAISGGFIRRVTNDARENEMDENLEQVSGIIGNLRHMALDMGNEIDTQNRQIDRIMEKADSNKTRIDEANQRATKMLGSG

SEQ ID NO: 15 - DNA, 981 bp, Artificial Sequence
  source: /note="Description of Artificial Sequence: Synthetic polynucleotide"
atggtcttcacactcgaagatttcgttggggactgggaacagacagccgcctacaacctggaccaagtccttgaacagggaggtgtgtccagtttgctgcagaatctcgccgtgtccgtaactccgatccaaaggattgtccggagcggtgaaaatgccctgaagatcgacatccatgtcatcatcccgtatgaaggtctgagcgccgaccaaatggcccagatcgaagaggtgtttaaggtggtgtaccctgtggatgatcatcactttaaggtgatcctgccctatggcacactggtaatcgacggggttacgccgaacatgctgaactatttcggacggccgtatgaaggcatcgccgtgttcgacggcaaaaagatcactgtaacagggaccctgtggaacggcaacaaaattatcgacgagcgcctgatcacccccgacggctccatgctgttccgagtaaccatcaacagtgggagttccggtggtggcgggagcggaggtggaggctcgagcggtggagctcagaacacctacttcaagaactgcacatttattgacactgtttttgacaacacagattttgagccatataaattcattgacagtgaatttaaaaactgctcgttttttcacaacaaggggggcggaggttccgcccgggaaaatgaaatggatgaaaacctagagcaggtgagcggcatcatcggaaacctccgtcatatggccctagacatgggcaatgagattgacacccagaatcgccagattgacaggatcatggagaaggctgactccaacaaaaccagaattgatgaagccaaccaacgtgcaacaaagatgctgggaagtggtgggaattctggctcgagcggtggtggcgggagcggaggtggagggtcgtcaggtgtgaccggctaccggctgttcgaggagattctggcggccgcactcgagcaccaccaccaccaccactga

SEQ ID NO: 16 - protein, 118 aa, Homo sapiens
MSAPAQPPAEGTEGTAPGGGPPGPPPNMTSNRRLQQTQAQVEEVVDIIRVNVDKVLERDQKLSELDDRADALQAGASQFESSAAKLKRKYWWKNCKMMIMLGAICAIIVVVIVIYFFT

SEQ ID NO: 17 - protein, 21 aa, Homo sapiens
GEGKEDAFSKLKQKFMNELHK

SEQ ID NO: 18 - protein, 21 aa, Homo sapiens
GESQEDMFAKLKEKFFNEINK

SEQ ID NO: 19 - protein, 28 aa, Homo sapiens
LSELDDRADALQAGASQFETSAAKLKRK

SEQ ID NO: 20 - protein, 28 aa, Homo sapiens
LSELDDRADALQAGASQFETSAAKLKRK

SEQ ID NO: 21 - protein, 28 aa, Homo sapiens
LSELDDRADALQAGASQFESSAAKLKRK

SEQ ID NO: 22 - skipped

SEQ ID NO: 23 - protein, 206 aa, Homo sapiens; identical to SEQ ID NO: 14

SEQ ID NO: 24 - protein, 118 aa, Homo sapiens; identical to SEQ ID NO: 16

SEQ ID NO: 25 - protein, 116 aa, Homo sapiens
MSATAATAPPAAPAGEGGPPAPPPNLTSNRRLQQTQAQVDEVVDIMRVNVDKVLERDQKLSELDDRADALQAGASQFETSAAKLKRKYWWKNLKMMIILGVICAIILIIIIVYFST

SEQ ID NO: 26 - protein, 100 aa, Homo sapiens
MSTGPTAATGSNRRLQQTQNQVDEVVDIMRVNVDKVLERDQKLSELDDRADALQAGASQFETSAAKLKRKYWWKNCKMWAIGITVLVIFIIIIIVWVVSS

SEQ ID NO: 27 - protein, 288 aa, Homo sapiens
MKDRTQELRTAKDSDDDDDVAVTVDRDRFMDEFFEQVEEIRGFIDKIAENVEEVKRKHSAILASPNPDEKTKEELEELMSDIKKTANKVRSKLKSIEQSIEQEEGLNRSSADLRIRKTQHSTLSRKFVEVMSEYNATQSDYRERCKGRIQRQLEITGRTTTSEELEDMLESGNPAIFASGIIMDSSISKQALSEIETRHSEIIKLENSIRELHDMFMDMAMLVESQGEMIDRIEYNVEHAVDYVERAVSDTKKAVKYQSKARRKKIMIIICCVILGIVIASTVGGIFA

SEQ ID NO: 28 - protein, 288 aa, Homo sapiens
MKDRTQELRSAKDSDDEEEVVHVDRDHFMDEFFEQVEEIRGCIEKLSEDVEQVKKQHSAILAAPNPDEKTKQELEDLTADIKKTANKVRSKLKAIEQSIEQEEGLNRSSADLRIRKTQHSTLSRKFVEVMTEYNATQSKYRDRCKDRIQRQLEITGRTTTNEELEDMLESGKLAIFTDDIKMDSQMTKQALNEIETRHNEIIKLETSIRELHDMFVDMAMLVESQGEMIDRIEYNVEHSVDYVERAVSDTKKAVKYQSKARRKKIMIIICCVVLGVVLASSIGGTLGL

SEQ ID NO: 29 - DNA, 852 bp, Artificial Sequence
  source: /note="Description of Artificial Sequence: Synthetic polynucleotide"
atggtcttcacactcgaagatttcgttggggactgggaacagacagccgcctacaacctggaccaagtccttgaacagggaggtgtgtccagtttgctgcagaatctcgccgtgtccgtaactccgatccaaaggattgtccggagcggtgaaaatgccctgaagatcgacatccatgtcatcatcccgtatgaaggtctgagcgccgaccaaatggcccagatcgaagaggtgtttaaggtggtgtaccctgtggatgatcatcactttaaggtgatcctgccctatggcacactggtaatcgacggggttacgccgaacatgctgaactatttcggacggccgtatgaaggcatcgccgtgttcgacggcaaaaagatcactgtaacagggaccctgtggaacggcaacaaaattatcgacgagcgcctgatcacccccgacggctccatgctgttccgagtaaccatcaacagtgggagttccggtggtggcgggagcggaggtggaggctcgagcggtggagctcaggcccgggaaaatgaaatggatgaaaacctagagcaggtgagcggcatcatcggaaacctccgtcatatggccctagacatgggcaatgagattgacacccagaatcgccagattgacaggatcatggagaaggctgactccaacaaaaccagaattgatgaagccaaccaacgtgcaacaaagatgctgggaagtggtgggaattctggctcgagcggtggtggcgggagcggaggtggagggtcgtcaggtgtgaccggctaccggctgttcgaggagattctggcggccgcactcgagcaccaccaccaccaccactga

SEQ ID NO: 30 - DNA, 840 bp, Artificial Sequence
  source: /note="Description of Artificial Sequence: Synthetic polynucleotide"
atggtcttcacactcgaagatttcgttggggactgggaacagacagccgcctacaacctggaccaagtccttgaacagggaggtgtgtccagtttgctgcagaatctcgccgtgtccgtaactccgatccaaaggattgtccggagcggtgaaaatgccctgaagatcgacatccatgtcatcatcccgtatgaaggtctgagcgccgaccaaatggcccagatcgaagaggtgtttaaggtggtgtaccctgtggatgatcatcactttaaggtgatcctgccctatggcacactggtaatcgacggggttacgccgaacatgctgaactatttcggacggccgtatgaaggcatcgccgtgttcgacggcaaaaagatcactgtaacagggaccctgtggaacggcaacaaaattatcgacgagcgcctgatcacccccgacggctccatgctgttccgagtaaccatcaacagtgggagttccggtggtggcgggagcggaggtggaggctcgagcggtggagctcagcagcaaacccaggcacaagtggaggaggtggtggacatcatacgtgtgaacgtggacaaggtcctggagagggaccagaagctgtcagagctggatgaccgagctgatgccttgcaggcaggagcatcacaatttgagagcagtgctgccaagctaaagaggaagtattggtggaaaaactgcaaggggaattctggctcgagcggtggtggcgggagcggaggtggagggtcgtcaggtgtgaccggctaccggctgttcgaggagattctggcggccgcactcgagcaccaccaccaccaccactga

SEQ ID NO: 31 - DNA, 2898 bp, Artificial Sequence
  source: /note="Description of Artificial Sequence: Synthetic polynucleotide"
atggtcttcacactcgaagatttcgttggggactgggaacagacagccgcctacaacctggaccaagtccttgaacagggaggtgtgtccagtttgctgcagaatctcgccgtgtccgtaactccgatccaaaggattgtccggagcggtgaaaatgccctgaagatcgacatccatgtcatcatcccgtatgaaggtctgagcgccgaccaaatggcccagatcgaagaggtgtttaaggtggtgtaccctgtggatgatcatcactttaaggtgatcctgccctatggcacactggtaatcgacggggttacgccgaacatgctgaactatttcggacggccgtatgaaggcatcgccgtgttcgacggcaaaaagatcactgtaacagggaccctgtggaacggcaacaaaattatcgacgagcgcctgatcacccccgacggctccatgctgttccgagtaaccatcaacagtgggagttccggtggtggcgggagcggaggtggaggctcgagcggtggagctcaggaagatgccaaaaacattaagaagggcccagcgccattctacccactcgaagacgggaccgccggcgagcagctgcacaaagccatgaagcgctacgccctggtgcccggcaccatcgcctttaccgacgcacatatcgaggtggacattacctacgccgagtacttcgagatgagcgttcggctggcagaagctatgaagcgctatgggctgaatacaaaccatcggatcgtggtgtgcagcgagaatagcttgcagttcttcatgcccgtgttgggtgccctgttcatcggtgtggctgtggccccagctaacgacatctacaacgagcgcgagctgctgaacagcatgggcatcagccagcccaccgtcgtattcgtgagcaagaaagggctgcaaaagatcctcaacgtgcaaaagaagctaccgatcatacaaaagatcatcatcatggatagcaagaccgactaccagggcttccaaagcatgtacaccttcgtgacttcccatttgccacccggcttcaacgagtacgacttcgtgcccgagagcttcgaccgggacaaaaccatcgccctgatcatgaacagtagtggcagtaccggattgcccaagggcgtagccctaccgcaccgcaccgcttgtgtccgattcagtcatgcccgcgaccccatcttcggcaaccagatcatccccgacaccgctatcctcagcgtggtgccatttcaccacggcttcggcatgttcaccacgctgggctacttgatctgcggctttcgggtcgtgctcatgtaccgcttcgaggaggagctattcttgcgcagcttgcaagactataagattcaatctgccctgctggtgcccacactatttagcttcttcgctaagagcactctcatcgacaagtacgacctaagcaacttgcacgagatcgccagcggcggggcgccgctcagcaaggaggtaggtgaggccgtggccaaacgcttccacctaccaggcatccgccagggctacggcctgacagaaacaaccagcgccattctgatcacccccgaaggggacgacaagcctggcgcagtaggcaaggtggtgcccttcttcgaggctaaggtggtggacttggacaccggtaagacactgggtgtgaaccagcgcggcgagctgtgcgtccgtggccccatgatcatgagcggctacgttaacaaccccgaggctacaaacgctctcatcgacaaggacggctggctgcacagcggcgacatcgcctactgggacgaggacgagcacttcttcatcgtggaccggctgaagagcctgatcaaatacaagggctaccaggtagccccagccgaactggagagcatcctgctgcaacaccccaacatcttcgacgccggggtcgccggcctgcccgacgacgatgccggcgagctgcccgccgcagtcgtcgtgctggaacacggtaaaaccatgaccgagaaggagatcgtggactatgtggccagccaggttacaaccgccaagaagctgcgcggtggtgttgtgttcgtggacgaggtgcctaaaggactgaccggcaagttggacgcccgcaagatccgcgagattctcattaaggccaagaagggcggcaagatcgccgtggggggcggaggttccgccgaggacgcagacatgcgtaatgaactggaggagatgcagaggagggctgaccagctggctgatgagtccctggaaagcacccgtcgcatgctgcagctggtcgaagagagtaaagatgctggcatcaggactttggttatgttggatgagcaaggcgaacaactggaacgcattgaggaagggatggaccaaatcaataaggatatgaaagaagcagaaaagaatttgacggacctaggaaaattctgcgggctttgtgtgtgtccctgtaacaagcttaaatccagtgatgcttacaaaaaagcctggggcaataatcaggatggagtagtggccagccagcctgcccgtgtggtggatgaacgggagcagatggccatcagtggtggcttcatccgcagggtaacaaacgatgcccgggaaaatgaaatggatgaaaacctagagcaggtgagcggcatcatcggaaacctccgtcatatggccctagacatgggcaatgagattgacacccagaatcgccagattgacaggatcatggagaaggctgactccaacaaaaccagaattgatgaagccaaccaacgtgcaacaaagatgctgggaagtggtgggaattctggctcgagcggtggtggcgggagcggaggtggagggtcgtcaggtgtgaccggctaccggctgttcgaggagattctgtaa

SEQ ID NO: 32 - protein, 15 aa, Artificial Sequence
  source: /note="Description of Artificial Sequence: Synthetic peptide"
GSSGGGGSGGGSSGG